European Patent Specification EP 3 811 080 B1, published February 11, 2026. Title: IN VITRO METHOD FOR THE DIAGNOSIS OF ECTOPIC PREGNANCY. Applicant: UNIVERSIDAD DE CORDOBA and FUNDACION IVI. The sequence listing filed with the application follows.

SEQUENCE LISTING (10 sequences)

SEQ ID NO: 1 - DNA, 19 bp, Artificial sequence
  Artificial sequence
agcagctagaatccctggg

SEQ ID NO: 2 - DNA, 19 bp, Artificial sequence
  Artificial sequence
aggccgaaggagttccagt

SEQ ID NO: 3 - DNA, 20 bp, Artificial sequence
  Artificial sequence
gaaatcgccaatgccaactc

SEQ ID NO: 4 - DNA, 20 bp, Artificial sequence
  Artificial sequence
accttcaggtacaggctgtg

SEQ ID NO: 5 - DNA, 24 bp, Artificial sequence
  Artificial sequence
ggagcttccaacccgaggcaataa

SEQ ID NO: 6 - DNA, 23 bp, Artificial sequence
  Artificial sequence
uuauugcuuaagaauacgcguag

SEQ ID NO: 7 - DNA, 23 bp, Artificial sequence
  Artificial sequence
gggcgcaggtgcggggcagtgaa

SEQ ID NO: 8 - DNA, 23 bp, Artificial sequence
  Artificial sequence
cccacugccccaggugcugcugg

SEQ ID NO: 9 - DNA, 14 bp, Artificial sequence
  Artificial sequence
ctgccttcagagac

SEQ ID NO: 10 - DNA, 21 bp, Artificial sequence
  Artificial sequence
cgucuugaaucggugacacuu